European Patent Application EP 4 663 755 A2, published December 17, 2025. Title: METHOD. Applicant: Hansa Biopharma AB. Application EP. The sequence listing filed with the application follows.

SEQUENCE LISTING (7 sequences)

SEQ ID NO: 1 - protein, 310 aa, Streptococcus pyogenes
DSFSANQEIRYSEVTPYHVTSVWTKGVTPPANFTQGEDVFHAPYVANQGWYDITKTFNGKDDLLCGAATAGNMLHWWFDQNKDQIKRYLEEHPEKQKINFNGEQMFDVKEAIDTKNHQLDSKLFEYFKEKAFPYLSTKHLGVFPDHVIDMFINGYRLSLTNHGPTPVKEGSKDPRGGIFDAVFTRGDQSKLLTSRHDFKEKNLKEISDLIKKELTEGKALGLSHTYANVRINHVINLWGADFDSNGNLKAIYVTDSDSNASIGMKKYFVGVNSAGKVAISAKEIKEDNIGAQVLGLFTLSTGQDSWNQTN

SEQ ID NO: 2 - protein, 959 aa, Streptococcus pyogenes
EEKTVQVQKGLPSIDSLHYLSENSKKEFKEELSKAGQESQKVKEILAKAQQADKQAQELAKMKIPEKIPMKPLHGPLYGGYFRTWHDKTSDPTEKDKVNSMGELPKEVDLAFIFHDWTKDYSLFWKELATKHVPKLNKQGTRVIRTIPWRFLAGGDNSGIAEDTSKYPNTPEGNKALAKAIVDEYVYKYNLDGLDVDVEHDSIPKVDKKEDTAGVERSIQVFEEIGKLIGPKGVDKSRLFIMDSTYMADKNPLIERGAPYINLLLVQVYGSQGEKGGWEPVSNRPEKTMEERWQGYSKYIRPEQYMIGFSFYEENAQEGNLWYDINSRKDEDKANGINTDITGTRAERYARWQPKTGGVKGGIFSYAIDRDGVAHQPKKYAKQKEFKDATDNIFHSDYSVSKALKTVMLKDKSYDLIDEKDFPDKALREAVMAQVGTRKGDLERFNGTLRLDNPAIQSLEGLNKFKKLAQLDLIGLSRITKLDRSVLPANMKPGKDTLETVLETYKKDNKEEPATIPPVSLKVSGLTGLKELDLSGFDRETLAGLDAATLTSLEKVDISGNKLDLAPGTENRQIFDTMLSTISNHVGSNEQTVKFDKQKPTGHYPDTYGKTSLRLPVANEKVDLQSQLLFGTVTNQGTLINSEADYKAYQNHKIAGRSFVDSNYHYNNFKVSYENYTVKVTDSTLGTTTDKTLATDKEETYKVDFFSPADKTKAVHTAKVIVGDEKTMMVNLAEGATVIGGSADPVNARKVFDGQLGSETDNISLGWDSKQSIIFKLKEDGLIKHWRFFNDSARNPETTNKPIQEASLQIFNIKDYNLDNLLENPNKFDDEKYWITVDTYSAQGERATAFSNTLNNITSKYWRVVFDTKGDRYSSPVVPELQILGYPLPNADTIMKTVTTAKELSQQKDKFSQKMLDELKIKEMALETSLNSKIFDVTAINANAGVLKDCIEKRQLLKK

SEQ ID NO: 3 - protein, 312 aa, Streptococcus pyogenes
DSFSANQEIRYSEVTPYHVTSVWTKGVTPPAKFTQGEDVFHAPYVANQGWYDITKTFNGKDDLLCGAATAGNMLHWWFDQNNEKIEAYLKKHPDKQKIMFGDQELLDVRKVINTKGDQTNSELFNYFRDKAFPGLSARRIGVMPDLVLDMFINGYYLNVYKTQTTDVNRTYQEKDRRGGIFDAVFTRGDQSKLLTSRHDFKEKTLKEISDLIKKELTEGKALGLSHTYANVRINHVINLWGADFDSNGNLEAIYVTDSDSNASIGMKKYFVGVNSAGKVAISAKEIKEDNIGAQVLGLFTLSTGQDSWNQTN

SEQ ID NO: 4 - protein, 6 aa, Streptococcus pyogenes
LFEYFK

SEQ ID NO: 5 - protein, 8 aa, Streptococcus pyogenes
AFPYLSTK

SEQ ID NO: 6 - protein, 16 aa, Streptococcus pyogenes
AIYVTDSDSNASIGMK

SEQ ID NO: 7 - protein, 10 aa, Streptococcus pyogenes
GGIFDAVFTR